European Patent Application EP 4 497 443 A1, published January 29, 2025. Title: Therapeutic/preventive agent targeting senescent cells or SASPs, methods for obtaining data for detecting senescent cells, and methods for screening therapeutic/preventive agent. Applicant: Japanese Foundation for Cancer Research. The sequence listing filed with the application follows.

SEQUENCE LISTING (12 sequences)

SEQ ID NO: 1 - RNA, 19 nt, synthetic construct
  misc_feature 1..19: note = siRNA
  source 1..19: mol_type = other RNA
tttccattccattccattc

SEQ ID NO: 2 - RNA, 19 nt, synthetic construct
  misc_feature 1..19: note = siRNA
  source 1..19: mol_type = other RNA
aatcatcgaatggtctcga

SEQ ID NO: 3 - RNA, 19 nt, synthetic construct
  misc_feature 1..19: note = siRNA control
  source 1..19: mol_type = other RNA
atgaacgtgaattgctcaa

SEQ ID NO: 4 - DNA, 20 bp, synthetic construct
  misc_feature 1..20: note = PCR primer
  source 1..20: mol_type = other DNA
aatcatcgaatggtctcgat

SEQ ID NO: 5 - DNA, 20 bp, synthetic construct
  misc_feature 1..20: note = PCR primer
  source 1..20: mol_type = other DNA
ataattccattcgattccac

SEQ ID NO: 6 - DNA, 20 bp, synthetic construct
  misc_feature 1..20: note = PCR primer
  source 1..20: mol_type = other DNA
ccagaatcgaaggccatcaa

SEQ ID NO: 7 - DNA, 24 bp, synthetic construct
  misc_feature 1..24: note = PCR primer
  source 1..24: mol_type = other DNA
catttccttgctaactgctttcag

SEQ ID NO: 8 - DNA, 19 bp, synthetic construct
  misc_feature 1..19: note = PCR primer
  source 1..19: mol_type = other DNA
aaccagtgctgctgaagga

SEQ ID NO: 9 - DNA, 21 bp, synthetic construct
  misc_feature 1..21: note = PCR primer
  source 1..21: mol_type = other DNA
ttcttagtgccgtgagtttcc

SEQ ID NO: 10 - DNA, 20 bp, synthetic construct
  misc_feature 1..20: note = PCR primer
  source 1..20: mol_type = other DNA
aaactcatgagcagtctgca

SEQ ID NO: 11 - DNA, 22 bp, synthetic construct
  misc_feature 1..22: note = PCR primer
  source 1..22: mol_type = other DNA
aggagatcttcagtttcggagg

SEQ ID NO: 12 - DNA, 291 bp, synthetic construct
  misc_feature 1..291: note = hSATII FISH probe
  source 1..291: mol_type = other DNA
aatcatcgaatgggcgttggaatcattatcaaatggaatcgaatggaatcaccgaatagaatcaaatggaacaatcatcgaatggactcaaatggaattatcctcaaatggaatcgaatggaattatcgaatgcaatcgaatggaattatcgaatgcaatcgaatagaatcatcgaatggactcgaatggaatcatcgaatggaatggaatggaaaactcaatgaactcgaatggaaccatcactgaatggaatcgaatggaatcatcgagtggaatcgaatggaattata